European Patent Specification EP 3 847 277 B1, published December 11, 2024. Title: Sequences and Their Use for Detection and Characterization of Escherichia coli Serotype O157:H7. Applicant: Hygiena, LLC Kalburge, Sai Wang, YangYang Padmalayam, Indira Martin, Easter. The sequence listing filed with the application follows.

SEQUENCE LISTING (13 sequences)

SEQ ID NO: 1 - DNA, 20 bp, Artificial Sequence
  Primer
ccgcgtgttacgtccgggct

SEQ ID NO: 2 - DNA, 20 bp, Artificial Sequence
  Primer
ttgcataggcgtcaccctga

SEQ ID NO: 3 - DNA, 20 bp, Artificial Sequence
  Primer
tgaaacccgcgtgttacgtc

SEQ ID NO: 4 - DNA, 20 bp, Artificial Sequence
  Primer
aggcgtcaccctgaccgtta

SEQ ID NO: 5 - DNA, 20 bp, Artificial Sequence
  Primer
gcgtgttacgtccgggctac

SEQ ID NO: 6 - DNA, 20 bp, Artificial Sequence
  Primer
gggtttgcataggcgtcacc

SEQ ID NO: 7 - DNA, 20 bp, Artificial Sequence
  Primer
gggctacgtcaagccgaaac

SEQ ID NO: 8 - DNA, 20 bp, Artificial Sequence
  Primer
gcataggcgtcaccctgacc

SEQ ID NO: 9 - DNA, 21 bp, Artificial Sequence
  Probe
tcaagccgaaacacgaattcc

SEQ ID NO: 10 - DNA, 22 bp, Artificial Sequence
  Probe
aattcccctggagccggtaaaa

SEQ ID NO: 11 - DNA, 21 bp, Artificial Sequence
  Probe
gaaacacgaattcccctggag

SEQ ID NO: 12 - DNA, 21 bp, Artificial Sequence
  Probe
gccggtaaaaggagccggtac

SEQ ID NO: 13 - DNA, 122 bp, Escherichia coli
tgaaacccgcgtgttacgtccgggctacgtcaagccgaaacacgaattcccctggagccggtaaaaggagccggtaccaccctgtgggtttataacggtcagggtgacgcctatgcaaaccc